European Patent Application EP 4 696 775 A1, published February 18, 2026. Title: Novel variant of (p)ppGpp synthetase and method for producing 5'-inosinic acid using the same. Applicant: DAESANG CORPORATION. The sequence listing filed with the application follows.

SEQUENCE LISTING (9 sequences)

SEQ ID NO: 1 - DNA, 2302 bp, synthetic construct
  source 1..2302: mol_type = other DNA
atgacgaacaataggtcaacgaaacgcccagccagcagtggcgttcgcagtatgtcggcccgcctcgcgcgttcgctgactgggggtcgcgtcaaggtcaatccagtccttgatccattgctgtctatccaccggcagtttcatcctcgcgctgacgtggaattgttaaacaatgcctattcgactgcggagatgctgcacgaaggggtatttcgcaagtcgggtgaaccttatatcacccacccattggcggtagcgacaattactgcggaaattggcatggacaccactactgtggtggcggcgctgctgcatgacacggttgaagacaccgattattcgctggatgacttaaccgctgatttcggccctgaagtcgctcgtctagttgatggagtgaccaaactggacaaggtagcccttggtgcggctgctgaagctgagaccatccgcaagatgattgtggcgatggctcatgacccacgcgtgctggtgattaaagttgctgaccgcttgcacaatatgcgcaccatgcgctttttgccgcccgaaaagcaggcgaagaaggcacgccaaacccttgatgtgattgcaccgcttgcgcaccgcttgggtatggcaaacgtgaagtgggagctagaggatctagcttttgccatcttgtacccaaagaaatatgacgagattgtccgcatggttgcagaccgtgcgccttcccgtgaccgtgctctggcagaaatcaaggatcaggtaagcggtgcgttgaaagaaaacggcattgacgctgaagtcatggggcggccgaagcactactggtctatttaccaaaagatgattgtgcgtggtcgcgactttgcggagatctttgacctcgtcggaatccgtatcttggttgatgacgtcaataattgctacgccgccattggtgttgtgcattcactcttccaggcgctgccaggcaggttcaaggactatatttccgcgcctcgttttggcgtgtatcagtcgctgcacaccaccgtgattgctggggaatccatcctagaagtgcaggtgcgtacgcacgagatgcactataacgcagaattcggcgttgctgcgcactggcgctacaaggagatgaagggtaagaactccggcaacagcgaagaagtcgatcagatggcgtggatgcgccagcttctggattggcaaaaagaagctgctgacccgaacgagttcttggactctttgcgctatgacttaacctcgcagcagatctttgcgtttacgcctaagggcgatgtggtgacgctgcctgcaggttcgaccccggtcgactttgcttatgccgtacacacggaggtaggccaccgttgtatcggtgcgaaggtcaacggcaagttggttgccttagaatcggagctaaagtccggtgacaaggtagaaatctttacctccaaagatgctaacgcaggtccatcgcgggactggcaggaatttcttgtctcgccgcgtgctaaggctaaggtacggcagtggtttgccaaagaacgccgagaagagcacttggaaaatggtcgtgatgcactagctactgaggtgcaacgcggtggtttgccaatgcaccggttgtttactgcttcgtcgatgaagcaggtagcagagcagctgcacttcgatgatgtcgatgctctctacacagccatcggcgcaggccacgtttctgcgcaacatgttgctaaccagctcatggctttgtttggcgatcgcgatgatgcagtggatgcgcttgcctcgcgcacgcctttgtcggaattggaaagctcacgcgcgaagcagcgcacgcagacggaggattccaaagctggtgccggcatcttggtggaaggaagccccgatgtgttggcgaagctcgccaagtgttgtcagccggttcctggagacgaaatctttggcttcgtaacccgcggcgggggagtctcggttcaccgtgcagactgtaccaacgcggataagctcaagagcgaaccagagcgcatggcgcaggttgagtgggaacaaggaaagtcgtcttccggtgctttcgctgcaaccttgcagctagaagcgctcgataggcaaggcctgctctttgaggtcaccaaggtatttaccgaagcgaagctgaacgtattatccatgcgctcggttcgaggtgaagaccatattgcgaccctgcagtttactttttcggtctcagataccaagcagcttgattctttgatgacaacgttgcgtaatactgaaggcgtattcgacgtctatcgcgtgactgcttagt

SEQ ID NO: 2 - protein, 766 aa, synthetic construct
MTNNRSTKRPASSGVRSMSARLARSLTGGRVKVNPVLDPLLSIHRQFHPRADVELLNNAYSTAEMLHEGVFRKSGEPYITHPLAVATITAEIGMDTTTVVAALLHDTVEDTDYSLDDLTADFGPEVARLVDGVTKLDKVALGAAAEAETIRKMIVAMAHDPRVLVIKVADRLHNMRTMRFLPPEKQAKKARQTLDVIAPLAHRLGMANVKWELEDLAFAILYPKKYDEIVRMVADRAPSRDRALAEIKDQVSGALKENGIDAEVMGRPKHYWSIYQKMIVRGRDFAEIFDLVGIRILVDDVNNCYAAIGVVHSLFQALPGRFKDYISAPRFGVYQSLHTTVIAGESILEVQVRTHEMHYNAEFGVAAHWRYKEMKGKNSGNSEEVDQMAWMRQLLDWQKEAADPNEFLDSLRYDLTSQQIFAFTPKGDVVTLPAGSTPVDFAYAVHTEVGHRCIGAKVNGKLVALESELKSGDKVEIFTSKDANAGPSRDWQEFLVSPRAKAKVRQWFAKERREEHLENGRDALATEVQRGGLPMHRLFTASSMKQVAEQLHFDDVDALYTAIGAGHVSAQHVANQLMALFGDRDDAVDALASRTPLSELESSRAKQRTQTEDSKAGAGILVEGSPDVLAKLAKCCQPVPGDEIFGFVTRGGGVSVHRADCTNADKLKSEPERMAQVEWEQGKSSSGAFAATLQLEALDRQGLLFEVTKVFTEAKLNVLSMRSVRGEDHIATLQFTFSVSDTKQLDSLMTTLRNTEGVFDVYRVTA

SEQ ID NO: 3 - DNA, 2302 bp, Corynebacterium stationis
  source 1..2302: mol_type = genomic DNA
atgacgaacaataggtcaacgaaacgcccagccagcagtggcgttcgcagtatgtcggcccgcctcgcgcgttcgctgactgggggtcgcgtcaaggtcaatccagtccttgatccattgctgtctatccaccggcagtttcatcctcgcgctgacgtggaattgttaaacaatgcctattcgactgcggagatgctgcacgaaggggtatttcgcaagtcgggtgaaccttatatcacccacccattggcggtagcgacaattactgcggaaattggcatggacaccactactgtggtggcggcgctgctgcatgacacggttgaagacaccgattattcgctggatgacttaaccgctgatttcggccctgaagtcgctcgtctagttgatggagtgaccaaactggacaaggtagcccttggtgcggctgctgaagctgagaccatccgcaagatgattgtggcgatggctcatgacccacgcgtgctggtgattaaagttgctgaccgcttgcacaatatgcgcaccatgcgctttttgccgcccgaaaagcaggcgaagaaggcacgccaaacccttgatgtgattgcaccgcttgcgcaccgcttgggtatggcaaacgtgaagtgggagctagaggatctagcttttgccatcttgtacccaaagaaatatgacgagattgtccgcatggttgcagaccgtgcgccttcccgtgaccgtgctctggcagaaatcaaggatcaggtaagcggtgcgttgaaagaaaacggcattgacgctgaagtcatggggcggccgaagcactactggtctatttaccaaaagatgattgtgcgtggtcgcgactttgcggagatctttgacctcgtcggaatccgtatcttggttgatgacgtcaataattgctacgccgccattggtgttgtgcattcactcttccaggcgctgccaggcaggttcaaggactatatttccgcgcctcgttttggcgtgtatcagtcgctgcacaccaccgtgattgctggggaatccatcctagaagtgcaggtgcgtacgcacgagatgcactataacgcagaattcggcgttgctgcgcactggcgctacaaggagatgaagggtaagaactccggcaacagcgaagaagtcgatcagatggcgtggatgcgccagcttctggattggcaaaaagaagctgctgacccgaacgagttcttggactctttgcgctatgacttaacctcgcagcagatctttgcgtttacgcctaagggcgatgtggtgacgctgcctgcaggttcgaccccggtcgactttgcttatgccgtacacacggaggtaggccaccgttgtatcggtgcgaaggtcaacggcaagttggttgccttagaatcggagctaaagtccggtgacaaggtagaaatctttacctccaaagatgctaacgcaggtccatcgcgggactggcaggaatttcttgtctcgccgcgtgctaaggctaaggtacggcagtggtttgccaaagaacgccgagaagagcacttggaaaatggtcgtgatgcactagctactgaggtgcaacgcggtggtttgccaatgcaccggttgtttactgcttcgtcgatgaagcaggtagcagagcagctgcacttcgatgatgtcgatgctctctacacagccatcggcgcaggccacgtttctgcgcaacatgttgctaaccagctcatggctttgtttggcgatcgcgatgatgcagtggatgcgcttgcctcgcgcacgcctttgtcggaattggaaagctcacgcgcgaagcagcgcacgcagacggaggattccaaagctggtgccggcatcttggtggaaggaagccccgatgtgttggcgaagctcgccaagtgttgtcagccggttcctggagacgaaatctttggcttcgtaacccgcggcgggggagtctcggttcaccgtgcagactgtaccaacgcggataagctcaagagcgaaccagagcgcatggcgcaggttgagtgggaacaaggaaagtcgtcttccggtgctttcgctgcaaccttgcagctagaagcgctcgataggcaaggcctgctctttgaggtcaccaaggtatttaccgaagcgaagctgaacgtattatccatgcgctcggttcgaggtgaagaccatattgcgaccctgcagtttactttttcggtctcagataccaagcagcttggttctttgatgacaacgttgcgtaatactgaaggcgtattcgacgtctatcgcgtgactgcttagt

SEQ ID NO: 4 - protein, 766 aa, Corynebacterium stationis
MTNNRSTKRPASSGVRSMSARLARSLTGGRVKVNPVLDPLLSIHRQFHPRADVELLNNAYSTAEMLHEGVFRKSGEPYITHPLAVATITAEIGMDTTTVVAALLHDTVEDTDYSLDDLTADFGPEVARLVDGVTKLDKVALGAAAEAETIRKMIVAMAHDPRVLVIKVADRLHNMRTMRFLPPEKQAKKARQTLDVIAPLAHRLGMANVKWELEDLAFAILYPKKYDEIVRMVADRAPSRDRALAEIKDQVSGALKENGIDAEVMGRPKHYWSIYQKMIVRGRDFAEIFDLVGIRILVDDVNNCYAAIGVVHSLFQALPGRFKDYISAPRFGVYQSLHTTVIAGESILEVQVRTHEMHYNAEFGVAAHWRYKEMKGKNSGNSEEVDQMAWMRQLLDWQKEAADPNEFLDSLRYDLTSQQIFAFTPKGDVVTLPAGSTPVDFAYAVHTEVGHRCIGAKVNGKLVALESELKSGDKVEIFTSKDANAGPSRDWQEFLVSPRAKAKVRQWFAKERREEHLENGRDALATEVQRGGLPMHRLFTASSMKQVAEQLHFDDVDALYTAIGAGHVSAQHVANQLMALFGDRDDAVDALASRTPLSELESSRAKQRTQTEDSKAGAGILVEGSPDVLAKLAKCCQPVPGDEIFGFVTRGGGVSVHRADCTNADKLKSEPERMAQVEWEQGKSSSGAFAATLQLEALDRQGLLFEVTKVFTEAKLNVLSMRSVRGEDHIATLQFTFSVSDTKQLGSLMTTLRNTEGVFDVYRVTA

SEQ ID NO: 5 - DNA, 5719 bp, synthetic construct
  source 1..5719: mol_type = other DNA
tgccgcaagcactcagggcgcaagggctgctaaaggaagcggaacacgtagaaagccagtccgcagaaacggtgctgaccccggatgaatgtcagctactgggctatctggacaagggaaaacgcaagcgcaaagagaaagcaggtagcttgcagtgggcttacatggcgatagctagactgggcggttttatggacagcaagcgaaccggaattgccagctggggcgccctctggtaaggttgggaagccctgcaaagtaaactggatggctttcttgccgccaaggatctgatggcgcaggggatcaagatctgatcaagagacaggatgaggatcgtttcgcatgattgaacaagatggattgcacgcaggttctccggccgcttgggtggagaggctattcggctatgactgggcacaacagacaatcggctgctctgatgccgccgtgttccggctgtcagcgcaggggcgcccggttctttttgtcaagaccgacctgtccggtgccctgaatgaactccaagacgaggcagcgcggctatcgtggctggccacgacgggcgttccttgcgcagctgtgctcgacgttgtcactgaagcgggaagggactggctgctattgggcgaagtgccggggcaggatctcctgtcatctcaccttgctcctgccgagaaagtatccatcatggctgatgcaatgcggcggctgcatacgcttgatccggctacctgcccattcgaccaccaagcgaaacatcgcatcgagcgagcacgtactcggatggaagccggtcttgtcgatcaggatgatctggacgaagagcatcaggggctcgcgccagccgaactgttcgccaggctcaaggcgcggatgcccgacggcgaggatctcgtcgtgacccatggcgatgcctgcttgccgaatatcatggtggaaaatggccgcttttctggattcatcgactgtggccggctgggtgtggcggaccgctatcaggacatagcgttggctacccgtgatattgctgaagagcttggcggcgaatgggctgaccgcttcctcgtgctttacggtatcgccgctcccgattcgcagcgcatcgccttctatcgccttcttgacgagttcttctgagcgggactctggggttcgctagaggatcgatcctttttaacccatcacatatacctgccgttcactattatttagtgaaatgagatattatgatattttctgaattgtgattaaaaaggcaactttatgcccatgcaacagaaactataaaaaatacagagaatgaaaagaaacagatagattttttagttctttaggcccgtagtctgcaaatccttttatgattttctatcaaacaaaagaggaaaatagaccagttgcaatccaaacgagagtctaatagaatgaggtcgaaaagtaaatcgcgcgggtttgttactgataaagcaggcaagacctaaaatgtgtaaagggcaaagtgtatactttggcgtcaccccttacatattttaggtctttttttattgtgcgtaactaacttgccatcttcaaacaggagggctggaagaagcagaccgctaacacagtacataaaaaaggagacatgaacgatgaacatcaaaaagtttgcaaaacaagcaacagtattaacctttactaccgcactgctggcaggaggcgcaactcaagcgtttgcgaaagaaacgaaccaaaagccatataaggaaacatacggcatttcccatattacacgccatgatatgctgcaaatccctgaacagcaaaaaaatgaaaaatatcaagtttctgaatttgattcgtccacaattaaaaatatctcttctgcaaaaggcctggacgtttgggacagctggccattacaaaacgctgacggcactgtcgcaaactatcacggctaccacatcgtctttgcattagccggagatcctaaaaatgcggatgacacatcgatttacatgttctatcaaaaagtcggcgaaacttctattgacagctggaaaaacgctggccgcgtctttaaagacagcgacaaattcgatgcaaatgattctatcctaaaagaccaaacacaagaatggtcaggttcagccacatttacatctgacggaaaaatccgtttattctacactgatttctccggtaaacattacggcaaacaaacactgacaactgcacaagttaacgtatcagcatcagacagctctttgaacatcaacggtgtagaggattataaatcaatctttgacggtgacggaaaaacgtatcaaaatgtacagcagttcatcgatgaaggcaactacagctcaggcgacaaccatacgctgagagatcctcactacgtagaagataaaggccacaaatacttagtatttgaagcaaacactggaactgaagatggctaccaaggcgaagaatctttatttaacaaagcatactatggcaaaagcacatcattcttccgtcaagaaagtcaaaaacttctgcaaagcgataaaaaacgcacggctgagttagcaaacggcgctctcggtatgattgagctaaacgatgattacacactgaaaaaagtgatgaaaccgctgattgcatctaacacagtaacagatgaaattgaacgcgcgaacgtctttaaaatgaacggcaaatggtacctgttcactgactcccgcggatcaaaaatgacgattgacggcattacgtctaacgatatttacatgcttggttatgtttctaattctttaactggcccatacaagccgctgaacaaaactggccttgtgttaaaaatggatcttgatcctaacgatgtaacctttacttactcacacttcgctgtacctcaagcgaaaggaaacaatgtcgtgattacaagctatatgacaaacagaggattctacgcagacaaacaatcaacgtttgcgccgagcttcctgctgaacatcaaaggcaagaaaacatctgttgtcaaagacagcatccttgaacaaggacaattaacagttaacaaataaaaacgcaaaagaaaatgccgatgggtaccgagcgaaatgaccgaccaagcgacgcccaacctgccatcacgagatttcgattccaccgccgccttctatgaaaggttgggcttcggaatcgttttccgggacgccctcgcggacgtgctcatagtccacgacgcccgtgattttgtagccctggccgacggccagcaggtaggccgacaggctcatgccggccgccgccgccttttcctcaatcgctcttcgttcgtctggaaggcagtacaccttgataggtgggctgcccttcctggttggcttggtttcatcagccatccgcttgccctcatctgttacgccggcggtagccggccagcctcgcagagcaggattcccgttgagcaccgccaggtgcgaataagggacagtgaagaaggaacacccgctcgcgggtgggcctacttcacctatcctgcccggctgacgccgttggatacaccaaggaaagtctacacgaaccctttggcaaaatcctgtatatcgtgcgaaaaaggatggatataccgaaaaaatcgctataatgaccccgaagcagggttatgcagcggaaaagcgctgcttccctgctgttttgtggaatatctaccgactggaaacaggcaaatgcaggaaattactgaactgaggggacaggcgagagacgatgccaaagagctcctgaaaatctcgataactcaaaaaatacgcccggtagtgatcttatttcattatggtgaaagttggaacctcttacgtgccgatcaacgtctcattttcgccaaaagttggcccagggcttcccggtatcaacagggacaccaggatttatttattctgcgaagtgatcttccgtcacaggtatttattcggcgcaaagtgcgtcgggtgatgctgccaacttactgatttagtgtatgatggtgtttttgaggtgctccagtggcttctgtttctatcagctcctgaaaatctcgataactcaaaaaatacgcccggtagtgatcttatttcattatggtgaaagttggaacctcttacgtgccgatcaacgtctcattttcgccaaaagttggcccagggcttcccggtatcaacagggacaccaggatttatttattctgcgaagtgatcttccgtcacaggtatttattcggcgcaaagtgcgtcgggtgatgctgccaacttactgatttagtgtatgatggtgtttttgaggtgctccagtggcttctgtttctatcagggctggatgatcctccagcgcggggatctcatgctggagttcttcgcccaccccaaaaggatctaggtgaagatcctttttgataatctcatgaccaaaatcccttaacgtgagttttcgttccactgagcgtcagaccccgtagaaaagatcaaaggatcttcttgagatcctttttttctgcgcgtaatctgctgcttgcaaacaaaaaaaccaccgctaccagcggtggtttgtttgccggatcaagagctaccaactctttttccgaaggtaactggcttcagcagagcgcagataccaaatactgttcttctagtgtagccgtagttaggccaccacttcaagaactctgtagcaccgcctacatacctcgctctgctaatcctgttaccagtggctgctgccagtggcgataagtcgtgtcttaccgggttggactcaagacgatagttaccggataaggcgcagcggtcgggctgaacggggggttcgtgcacacagcccagcttggagcgaacgacctacaccgaactgagatacctacagcgtgagctatgagaaagcgccacgcttcccgaagggagaaaggcggacaggtatccggtaagcggcagggtcggaacaggagagcgcacgagggagcttccagggggaaacgcctggtatctttatagtcctgtcgggtttcgccacctctgacttgagcgtcgatttttgtgatgctcgtcaggggggcggagcctatggaaaaacgccagcaacgcggcctttttacggttcctggccttttgctggccttttgctcacatgttctttcctgcgttatcccctgattctgtggataaccgtattaccgcctttgagtgagctgataccgctcgccgcagccgaacgaccgagcgcagcgagtcagtgagcgaggaagcggaagagcgcccaatacgcaaaccgcctctccccgcgcgttggccgattcattaatgcagctggcacgacaggtttcccgactggaaagcgggcagtgagcgcaacgcaattaatgtgagttagctcactcattaggcaccccaggctttacactttatgcttccggctcgtatgttgtgtggaattgtgagcggataacaatttcacacaggaaacagctatgacatgattacgccaagcttgcatgcctgcaggtcgactctagaggatccccgggtaccgagctcgaattcactggccgtcgttttacaacgtcgtgactgggaaaaccctggcgttacccaacttaatcgccttgcagcacatccccctttcgccagctggcgtaatagcgaagaggcccgcaccgatcgcccttcccaacagttgcgcagcctgaatggcgaatggcgataagctagcttcacgc

SEQ ID NO: 6 - DNA, 20 bp, synthetic construct
  source 1..20: mol_type = other DNA
tgatgcagtggatgcgcttg

SEQ ID NO: 7 - DNA, 29 bp, synthetic construct
  source 1..29: mol_type = other DNA
tgtcatcaaagaatcaagctgcttggtat

SEQ ID NO: 8 - DNA, 28 bp, synthetic construct
  source 1..28: mol_type = other DNA
taccaagcagcttgattctttgatgaca

SEQ ID NO: 9 - DNA, 25 bp, synthetic construct
  source 1..25: mol_type = other DNA
ggaggtagtcatgatgtattcctgg